European Patent Application EP 4 644 411 A1, published November 5, 2025. Title: CHIMERIC AUTOANTIGEN RECEPTOR FOR TREATING AUTOIMMUNE DISEASE. Applicant: ISAR Bioscience GmbH. The sequence listing filed with the application follows.

SEQUENCE LISTING (17 sequences)

SEQ ID NO: 1 - protein, 413 aa, synthetic construct
MRPADLLQLVLLLDLPRDLGGMGCSSPPCECHQEEDFRVTCKDIQRIPSLPPSTQTLKLIETHLRTIPSHAFSNLPNISRIYVSIDVTLQQLESHSFYNLSKVTHIEIRNTRNLTYIDPDALKELPLLKFLGIFNTGLKMFPDLTKVYSTDIFFILEITDNPYMTSIPVNAFQGLCNETLTLKLYNNGFTSVQGYAFNGTKLDAVYLNKNKYLTVIDKDAFGGVYSGPSLLDVSQTSVTALPSKGLEHLKELIARNTWTLKKLPLSLSFLHLTRADLSYPSHCCAFKNQKKIRGILESLMCNESSMQSLRQRKSVNALNSPLHQEYEENLGDSIVGYKEKSKFQDTHNNAHYYVFFEEQEDEIIGFGQELKNPQEETLQAFDSHYDYTICGDSEDMVCTPKSDEFNPCEDIMG

SEQ ID NO: 2 - DNA, 1239 bp, synthetic construct
  source 1..1239: mol_type = other DNA
atgaggccggcggacttgctgcagctggtgctgctgctcgacctgcccagggacctgggcggaatggggtgttcgtctccaccctgcgagtgccatcaggaggaggacttcagagtcacctgcaaggatattcaacgcatccccagcttaccgcccagtacgcagactctgaagcttattgagactcacctgagaactattccaagtcatgcattttctaatctgcccaatatttccagaatctacgtatctatagatgtgactctgcagcagctggaatcacactccttctacaatttgagtaaagtgactcacatagaaattcggaataccaggaacttaacttacatagaccctgatgccctcaaagagctccccctcctaaagttccttggcattttcaacactggacttaaaatgttccctgacctgaccaaagtttattccactgatatattctttatacttgaaattacagacaacccttacatgacgtcaatccctgtgaatgcttttcagggactatgcaatgaaaccttgacactgaagctgtacaacaatggctttacttcagtccaaggatatgctttcaatgggacaaagctggatgctgtttacctaaacaagaataaatacctgacagttattgacaaagatgcatttggaggagtatacagtggaccaagcttgctggacgtgtctcaaaccagtgtcactgcccttccatccaaaggcctggagcacctgaaggaactgatagcaagaaacacctggactcttaagaaacttccactttccttgagtttccttcacctcacacgggctgacctttcttacccaagccactgctgtgcttttaagaatcagaagaaaatcagaggaatccttgagtccttgatgtgtaatgagagcagtatgcagagcttgcgccagagaaaatctgtgaatgccttgaatagccccctccaccaggaatatgaagagaatctgggtgacagcattgttgggtacaaggaaaagtccaagttccaggatactcataacaacgctcattattacgtcttctttgaagaacaagaggatgagatcattggttttggccaggagctcaaaaacccccaggaagagactctacaagcttttgacagccattatgactacaccatatgtggggacagtgaagacatggtgtgtacccccaagtccgatgagttcaacccgtgtgaagacataatgggc

SEQ ID NO: 3 - protein, 48 aa, synthetic construct
AKPTTTPAPRPPTPAPTIASQPLSLRPEACRPAAGGAVHTRGLDFACD

SEQ ID NO: 4 - DNA, 144 bp, synthetic construct
  source 1..144: mol_type = other DNA
gcgaagcccaccacgacgccagcgccgcgaccaccaacaccggcgcccaccatcgcgtcgcagcccctgtccctgcgcccagaggcgtgccggccagcggcggggggcgcagtgcacacgagggggctggacttcgcctgtgat

SEQ ID NO: 5 - protein, 24 aa, synthetic construct
IYIWAPLAGTCGVLLLSLVITLYC

SEQ ID NO: 6 - DNA, 72 bp, synthetic construct
  source 1..72: mol_type = other DNA
atctacatctgggcgcccttggccgggacttgtggggtccttctcctgtcactggttatcaccctttactgc

SEQ ID NO: 7 - protein, 42 aa, synthetic construct
KRGRKKLLYIFKQPFMRPVQTTQEEDGCSCRFPEEEEGGCEL

SEQ ID NO: 8 - DNA, 126 bp, synthetic construct
  source 1..126: mol_type = other DNA
aaacggggcagaaagaaactcctgtatatattcaaacaaccatttatgagaccagtacaaactactcaagaggaagatggctgtagctgccgatttccagaagaagaagaaggaggatgtgaactg

SEQ ID NO: 9 - protein, 112 aa, synthetic construct
RVKFSRSADAPAYQQGQNQLYNELNLGRREEYDVLDKRRGRDPEMGGKPRRKNPQEGLYNELQKDKMAEAYSEIGMKGERRRGKGHDGLYQGLSTATKDTYDALHMQALPPR

SEQ ID NO: 10 - DNA, 336 bp, synthetic construct
  source 1..336: mol_type = other DNA
agagtgaagttcagcaggagcgcagacgcccccgcgtaccagcagggccagaaccagctctataacgagctcaatctaggacgaagagaggagtacgatgttttggacaagagacgtggccgggaccctgagatggggggaaagccgagaaggaagaaccctcaggaaggcctgtacaatgaactgcagaaagataagatggcggaggcctacagtgagattgggatgaaaggcgagcgccggaggggcaaggggcacgatggcctttaccagggtctcagtacagccaccaaggacacctacgacgcccttcacatgcaggccctgccccctcgc

SEQ ID NO: 11 - protein, 21 aa, synthetic construct
MALPVTALLLPLALLLHAARP

SEQ ID NO: 12 - DNA, 63 bp, synthetic construct
  source 1..63: mol_type = other DNA
atggccttaccagtgaccgccttgctcctgccgctggccttgctgctccacgccgccaggccg

SEQ ID NO: 13 - protein, 515 aa, synthetic construct
MALPVTALLLPLALLLHAARPMGCSSPPCECHQEEDFRVTCKDIQRIPSLPPSTQTLKLIETHLRTIPSHAFSNLPNISRIYVSIDVTLQQLESHSFYNLSKVTHIEIRNTRNLTYIDPDALKELPLLKFLGIFNTGLKMFPDLTKVYSTDIFFILEITDNPYMTSIPVNAFQGLCNETLTLKLYNNGFTSVQGYAFNGTKLDAVYLNKNKYLTVIDKDAFGGVYSGPSLLDVSQTSVTALPSKGLEHLKELIARNTWTLKKLPLSLSFLHLTRADLSYPSHCCAFKNQAKPTTTPAPRPPTPAPTIASQPLSLRPEACRPAAGGAVHTRGLDFACDIYIWAPLAGTCGVLLLSLVITLYCKRGRKKLLYIFKQPFMRPVQTTQEEDGCSCRFPEEEEGGCELRVKFSRSADAPAYQQGQNQLYNELNLGRREEYDVLDKRRGRDPEMGGKPRRKNPQEGLYNELQKDKMAEAYSEIGMKGERRRGKGHDGLYQGLSTATKDTYDALHMQALPPR

SEQ ID NO: 14 - DNA, 1548 bp, synthetic construct
  source 1..1548: mol_type = other DNA
atggccttaccagtgaccgccttgctcctgccgctggccttgctgctccacgccgccaggccgatgggatgtagctctccaccttgcgagtgccaccaagaagaggacttccgggtcacatgcaaggacatccagagaatccccagcctgcctcctagcacacagaccctgaagctgatcgagacacacctgagaacaatccctagccacgccttctccaacctgcctaacatctcccggatctacgtgtccatcgacgtgaccctgcagcagctggaatcccacagcttctacaacctgtccaaagtgacccacatcgagatccggaacacccggaacctgacctacatcgaccccgacgctctgaaagagctgcccctgctgaagttcctgggcatcttcaacaccggcctgaagatgttccccgacctgaccaaggtgtactctaccgacatcttcttcatcctggaaatcacagacaacccctacatgaccagcattcccgtgaacgccttccagggcctgtgcaacgaaaccctgacactgaagctgtacaacaacggcttcacctccgtgcagggctacgccttcaatggcaccaagctggatgccgtgtacctgaacaagaacaagtacctgaccgtgatcgacaaggacgccttcggcggagtgtactctggaccttctctgctggatgtgtcccagacctctgtgaccgctctgccctctaaaggcctggaacacctgaaagaactgatcgcccggaacacatggactctgaagaagctgcctctgagcctgtccttcctgcacctgaccagagccgacctgagctacccttctcactgctgcgccttcaagaaccaggcgaagcccaccacgacgccagcgccgcgaccaccaacaccggcgcccaccatcgcgtcgcagcccctgtccctgcgcccagaggcgtgccggccagcggcggggggcgcagtgcacacgagggggctggacttcgcctgtgatatctacatctgggcgcccttggccgggacttgtggggtccttctcctgtcactggttatcaccctttactgcaaacggggcagaaagaaactcctgtatatattcaaacaaccatttatgagaccagtacaaactactcaagaggaagatggctgtagctgccgatttccagaagaagaagaaggaggatgtgaactgagagtgaagttcagcaggagcgcagacgcccccgcgtaccagcagggccagaaccagctctataacgagctcaatctaggacgaagagaggagtacgatgttttggacaagagacgtggccgggaccctgagatggggggaaagccgagaaggaagaaccctcaggaaggcctgtacaatgaactgcagaaagataagatggcggaggcctacagtgagattgggatgaaaggcgagcgccggaggggcaaggggcacgatggcctttaccagggtctcagtacagccaccaaggacacctacgacgcccttcacatgcaggccctgccccctcgctaa

SEQ ID NO: 15 - protein, 268 aa, synthetic construct
MGCSSPPCECHQEEDFRVTCKDIQRIPSLPPSTQTLKLIETHLRTIPSHAFSNLPNISRIYVSIDVTLQQLESHSFYNLSKVTHIEIRNTRNLTYIDPDALKELPLLKFLGIFNTGLKMFPDLTKVYSTDIFFILEITDNPYMTSIPVNAFQGLCNETLTLKLYNNGFTSVQGYAFNGTKLDAVYLNKNKYLTVIDKDAFGGVYSGPSLLDVSQTSVTALPSKGLEHLKELIARNTWTLKKLPLSLSFLHLTRADLSYPSHCCAFKNQ

SEQ ID NO: 16 - DNA, 804 bp, synthetic construct
  source 1..804: mol_type = other DNA
atgggatgtagctctccaccttgcgagtgccaccaagaagaggacttccgggtcacatgcaaggacatccagagaatccccagcctgcctcctagcacacagaccctgaagctgatcgagacacacctgagaacaatccctagccacgccttctccaacctgcctaacatctcccggatctacgtgtccatcgacgtgaccctgcagcagctggaatcccacagcttctacaacctgtccaaagtgacccacatcgagatccggaacacccggaacctgacctacatcgaccccgacgctctgaaagagctgcccctgctgaagttcctgggcatcttcaacaccggcctgaagatgttccccgacctgaccaaggtgtactctaccgacatcttcttcatcctggaaatcacagacaacccctacatgaccagcattcccgtgaacgccttccagggcctgtgcaacgaaaccctgacactgaagctgtacaacaacggcttcacctccgtgcagggctacgccttcaatggcaccaagctggatgccgtgtacctgaacaagaacaagtacctgaccgtgatcgacaaggacgccttcggcggagtgtactctggaccttctctgctggatgtgtcccagacctctgtgaccgctctgccctctaaaggcctggaacacctgaaagaactgatcgcccggaacacatggactctgaagaagctgcctctgagcctgtccttcctgcacctgaccagagccgacctgagctacccttctcactgctgcgccttcaagaaccag

SEQ ID NO: 17 - protein, 11348 aa, synthetic construct
AATGTAGTCTTATGCAATACTCTTGTAGTCTTGCAACATGGTAACGATGAGTTAGCAACATGCCTTACAAGGAGAGAAAAAGCACCGTGCATGCCGATTGGTGGAAGTAAGGTGGTACGATCGTGCCTTATTAGGAAGGCAACAGACGGGTCTGACATGGATTGGACGAACCACTGAATTGCCGCATTGCAGAGATATTGTATTTAAGTGCCTAGCTCGATACATAAACGGGTCTCTCTGGTTAGACCAGATCTGAGCCTGGGAGCTCTCTGGCTAACTAGGGAACCCACTGCTTAAGCCTCAATAAAGCTTGCCTTGAGTGCTTCAAGTAGTGTGTGCCCGTCTGTTGTGTGACTCTGGTAACTAGAGATCCCTCAGACCCTTTTAGTCAGTGTGGAAAATCTCTAGCAGTGGCGCCCGAACAGGGACTTGAAAGCGAAAGGGAAACCAGAGGAGCTCTCTCGACGCAGGACTCGGCTTGCTGAAGCGCGCACGGCAAGAGGCGAGGGGCGGCGACTGGTGAGTACGCCAAAAATTTTGACTAGCGGAGGCTAGAAGGAGAGAGATGGGTGCGAGAGCGTCAGTATTAAGCGGGGGAGAATTAGATCGCGATGGGAAAAAATTCGGTTAAGGCCAGGGGGAAAGAAAAAATATAAATTAAAACATATAGTATGGGCAAGCAGGGAGCTAGAACGATTCGCAGTTAATCCTGGCCTGTTAGAAACATCAGAAGGCTGTAGACAAATACTGGGACAGCTACAACCATCCCTTCAGACAGGATCAGAAGAACTTAGATCATTATATAATACAGTAGCAACCCTCTATTGTGTGCATCAAAGGATAGAGATAAAAGACACCAAGGAAGCTTTAGACAAGATAGAGGAAGAGCAAAACAAAAGTAAGACCACCGCACAGCAAGCGGCCGCTGATCTTCAGACCTGGAGGAGGAGATATGAGGGACAATTGGAGAAGTGAATTATATAAATATAAAGTAGTAAAAATTGAACCATTAGGAGTAGCACCCACCAAGGCAAAGAGAAGAGTGGTGCAGAGAGAAAAAAGAGCAGTGGGAATAGGAGCTTTGTTCCTTGGGTTCTTGGGAGCAGCAGGAAGCACTATGGGCGCAGCGTCAATGACGCTGACGGTACAGGCCAGACAATTATTGTCTGGTATAGTGCAGCAGCAGAACAATTTGCTGAGGGCTATTGAGGCGCAACAGCATCTGTTGCAACTCACAGTCTGGGGCATCAAGCAGCTCCAGGCAAGAATCCTGGCTGTGGAAAGATACCTAAAGGATCAACAGCTCCTGGGGATTTGGGGTTGCTCTGGAAAACTCATTTGCACCACTGCTGTGCCTTGGAATGCTAGTTGGAGTAATAAATCTCTGGAACAGATTTGGAATCACACGACCTGGATGGAGTGGGACAGAGAAATTAACAATTACACAAGCTTAATACACTCCTTAATTGAAGAATCGCAAAACCAGCAAGAAAAGAATGAACAAGAATTATTGGAATTAGATAAATGGGCAAGTTTGTGGAATTGGTTTAACATAACAAATTGGCTGTGGTATATAAAATTATTCATAATGATAGTAGGAGGCTTGGTAGGTTTAAGAATAGTTTTTGCTGTACTTTCTATAGTGAATAGAGTTAGGCAGGGATATTCACCATTATCGTTTCAGACCCACCTCCCAACCCCGAGGGGACCCGACAGGCCCGAAGGAATAGAAGAAGAAGGTGGAGAGAGAGACAGAGACAGATCCATTCGATTAGTGAACGGATCTCGACGGTATCGCTAGCTTTTAAAAGAAAAGGGGGGATTGGGGGGTACAGTGCAGGGGAAAGAATAGTAGACATAATAGCAACAGACATACAAACTAAAGAATTACAAAAACAAATTACAAAAATTCAAAATTTTACTAGTGATTATCGGATCAACTTTGTATAGAAAAGTTGGGCTCCGGTGCCCGTCAGTGGGCAGAGCGCACATCGCCCACAGTCCCCGAGAAGTTGGGGGGAGGGGTCGGCAATTGAACCGGTGCCTAGAGAAGGTGGCGCGGGGTAAACTGGGAAAGTGATGTCGTGTACTGGCTCCGCCTTTTTCCCGAGGGTGGGGGAGAACCGTATATAAGTGCAGTAGTCGCCGTGAACGTTCTTTTTCGCAACGGGTTTGCCGCCAGAACACAGGTAAGTGCCGTGTGTGGTTCCCGCGGGCCTGGCCTCTTTACGGGTTATGGCCCTTGCGTGCCTTGAATTACTTCCACCTGGCTGCAGTACGTGATTCTTGATCCCGAGCTTCGGGTTGGAAGTGGGTGGGAGAGTTCGAGGCCTTGCGCTTAAGGAGCCCCTTCGCCTCGTGCTTGAGTTGAGGCCTGGCCTGGGCGCTGGGGCCGCCGCGTGCGAATCTGGTGGCACCTTCGCGCCTGTCTCGCTGCTTTCGATAAGTCTCTAGCCATTTAAAATTTTTGATGACCTGCTGCGACGCTTTTTTTCTGGCAAGATAGTCTTGTAAATGCGGGCCAAGATCTGCACACTGGTATTTCGGTTTTTGGGGCCGCGGGCGGCGACGGGGCCCGTGCGTCCCAGCGCACATGTTCGGCGAGGCGGGGCCTGCGAGCGCGGCCACCGAGAATCGGACGGGGGTAGTCTCAAGCTGGCCGGCCTGCTCTGGTGCCTGGTCTCGCGCCGCCGTGTATCGCCCCGCCCTGGGCGGCAAGGCTGGCCCGGTCGGCACCAGTTGCGTGAGCGGAAAGATGGCCGCTTCCCGGCCCTGCTGCAGGGAGCTCAAAATGGAGGACGCGGCGCTCGGGAGAGCGGGCGGGTGAGTCACCCACACAAAGGAAAAGGGCCTTTCCGTCCTCAGCCGTCGCTTCATGTGACTCCACGGAGTACCGGGCGCCGTCCAGGCACCTCGATTAGTTCTCGAGCTTTTGGAGTACGTCGTCTTTAGGTTGGGGGGAGGGGTTTTATGCGATGGAGTTTCCCCACACTGAGTGGGTGGAGACTGAAGTTAGGCCAGCTTGGCACTTGATGTAATTCTCCTTGGAATTTGCCCTTTTTGAGTTTGGATCTTGGTTCATTCTCAAGCCTCAGACAGTGGTTCAAAGTTTTTTTCTTCCATTTCAGGTGTCGTGACAAGTTTGTACAAAAAAGCAGGCTGCCACCATGGCCTTACCAGTGACCGCCTTGCTCCTGCCGCTGGCCTTGCTGCTCCACGCCGCCAGGCCGATGGGATGTAGCTCTCCACCTTGCGAGTGCCACCAAGAAGAGGACTTCCGGGTCACATGCAAGGACATCCAGAGAATCCCCAGCCTGCCTCCTAGCACACAGACCCTGAAGCTGATCGAGACACACCTGAGAACAATCCCTAGCCACGCCTTCTCCAACCTGCCTAACATCTCCCGGATCTACGTGTCCATCGACGTGACCCTGCAGCAGCTGGAATCCCACAGCTTCTACAACCTGTCCAAAGTGACCCACATCGAGATCCGGAACACCCGGAACCTGACCTACATCGACCCCGACGCTCTGAAAGAGCTGCCCCTGCTGAAGTTCCTGGGCATCTTCAACACCGGCCTGAAGATGTTCCCCGACCTGACCAAGGTGTACTCTACCGACATCTTCTTCATCCTGGAAATCACAGACAACCCCTACATGACCAGCATTCCCGTGAACGCCTTCCAGGGCCTGTGCAACGAAACCCTGACACTGAAGCTGTACAACAACGGCTTCACCTCCGTGCAGGGCTACGCCTTCAATGGCACCAAGCTGGATGCCGTGTACCTGAACAAGAACAAGTACCTGACCGTGATCGACAAGGACGCCTTCGGCGGAGTGTACTCTGGACCTTCTCTGCTGGATGTGTCCCAGACCTCTGTGACCGCTCTGCCCTCTAAAGGCCTGGAACACCTGAAAGAACTGATCGCCCGGAACACATGGACTCTGAAGAAGCTGCCTCTGAGCCTGTCCTTCCTGCACCTGACCAGAGCCGACCTGAGCTACCCTTCTCACTGCTGCGCCTTCAAGAACCAGGCGAAGCCCACCACGACGCCAGCGCCGCGACCACCAACACCGGCGCCCACCATCGCGTCGCAGCCCCTGTCCCTGCGCCCAGAGGCGTGCCGGCCAGCGGCGGGGGGCGCAGTGCACACGAGGGGGCTGGACTTCGCCTGTGATATCTACATCTGGGCGCCCTTGGCCGGGACTTGTGGGGTCCTTCTCCTGTCACTGGTTATCACCCTTTACTGCAAACGGGGCAGAAAGAAACTCCTGTATATATTCAAACAACCATTTATGAGACCAGTACAAACTACTCAAGAGGAAGATGGCTGTAGCTGCCGATTTCCAGAAGAAGAAGAAGGAGGATGTGAACTGAGAGTGAAGTTCAGCAGGAGCGCAGACGCCCCCGCGTACCAGCAGGGCCAGAACCAGCTCTATAACGAGCTCAATCTAGGACGAAGAGAGGAGTACGATGTTTTGGACAAGAGACGTGGCCGGGACCCTGAGATGGGGGGAAAGCCGAGAAGGAAGAACCCTCAGGAAGGCCTGTACAATGAACTGCAGAAAGATAAGATGGCGGAGGCCTACAGTGAGATTGGGATGAAAGGCGAGCGCCGGAGGGGCAAGGGGCACGATGGCCTTTACCAGGGTCTCAGTACAGCCACCAAGGACACCTACGACGCCCTTCACATGCAGGCCCTGCCCCCTCGCTAAACCCAGCTTTCTTGTACAAAGTGGTGATAATCGAATTCCGATAATCAACCTCTGGATTACAAAATTTGTGAAAGATTGACTGGTATTCTTAACTATGTTGCTCCTTTTACGCTATGTGGATACGCTGCTTTAATGCCTTTGTATCATGCTATTGCTTCCCGTATGGCTTTCATTTTCTCCTCCTTGTATAAATCCTGGTTGCTGTCTCTTTATGAGGAGTTGTGGCCCGTTGTCAGGCAACGTGGCGTGGTGTGCACTGTGTTTGCTGACGCAACCCCCACTGGTTGGGGCATTGCCACCACCTGTCAGCTCCTTTCCGGGACTTTCGCTTTCCCCCTCCCTATTGCCACGGCGGAACTCATCGCCGCCTGCCTTGCCCGCTGCTGGACAGGGGCTCGGCTGTTGGGCACTGACAATTCCGTGGTGTTGTCGGGGAAGCTGACGTCCTTTCCATGGCTGCTCGCCTGTGTTGCCACCTGGATTCTGCGCGGGACGTCCTTCTGCTACGTCCCTTCGGCCCTCAATCCAGCGGACCTTCCTTCCCGCGGCCTGCTGCCGGCTCTGCGGCCTCTTCCGCGTCTTCGCCTTCGCCCTCAGACGAGTCGGATCTCCCTTTGGGCCGCCTCCCCGCATCGGGAATTCCCGCGGTTCGAACGCGTTGACATTGATTATTGACTAGTTATTAATAGTAATCAATTACGGGGTCATTAGTTCATAGCCCATATATGGAGTTCCGCGTTACATAACTTACGGTAAATGGCCCGCCTGGCTGACCGCCCAACGACCCCCGCCCATTGACGTCAATAATGACGTATGTTCCCATAGTAACGCCAATAGGGACTTTCCATTGACGTCAATGGGTGGAGTATTTACGGTAAACTGCCCACTTGGCAGTACATCAAGTGTATCATATGCCAAGTACGCCCCCTATTGACGTCAATGACGGTAAATGGCCCGCCTGGCATTATGCCCAGTACATGACCTTATGGGACTTTCCTACTTGGCAGTACATCTACGTATTAGTCATCGCTATTACCATGGTGATGCGGTTTTGGCAGTACATCAATGGGCGTGGATAGCGGTTTGACTCACGGGGATTTCCAAGTCTCCACCCCATTGACGTCAATGGGAGTTTGTTTTGGCACCAAAATCAACGGGACTTTCCAAAATGTCGTAACAACTCCGCCCCATTGACGCAAATGGGCGGTAGGCGTGTACGGTGGGAGGTCTATATAAGCAGAGCTCTCTGGCTAACTAGAGAACCCACTGCGCCACCATGGTGAGCAAGGGCGAGGAGCTGTTCACCGGGGTGGTGCCCATCCTGGTCGAGCTGGACGGCGACGTAAACGGCCACAAGTTCAGCGTGTCCGGCGAGGGCGAGGGCGATGCCACCTACGGCAAGCTGACCCTGAAGTTCATCTGCACCACCGGCAAGCTGCCCGTGCCCTGGCCCACCCTCGTGACCACCCTGACCTACGGCGTGCAGTGCTTCAGCCGCTACCCCGACCACATGAAGCAGCACGACTTCTTCAAGTCCGCCATGCCCGAAGGCTACGTCCAGGAGCGCACCATCTTCTTCAAGGACGACGGCAACTACAAGACCCGCGCCGAGGTGAAGTTCGAGGGCGACACCCTGGTGAACCGCATCGAGCTGAAGGGCATCGACTTCAAGGAGGACGGCAACATCCTGGGGCACAAGCTGGAGTACAACTACAACAGCCACAACGTCTATATCATGGCCGACAAGCAGAAGAACGGCATCAAGGTGAACTTCAAGATCCGCCACAACATCGAGGACGGCAGCGTGCAGCTCGCCGACCACTACCAGCAGAACACCCCCATCGGCGACGGCCCCGTGCTGCTGCCCGACAACCACTACCTGAGCACCCAGTCCGCCCTGAGCAAAGACCCCAACGAGAAGCGCGATCACATGGTCCTGCTGGAGTTCGTGACCGCCGCCGGGATCACTCTCGGCATGGACGAGCTGTACAAGGGCTCCGGAGAGGGCAGGGGAAGTCTTCTAACATGCGGGGACGTGGAGGAAAATCCCGGCCCCATGAAAAAGCCTGAACTCACCGCGACGTCTGTCGAGAAGTTTCTGATCGAAAAGTTCGACAGCGTCTCCGACCTGATGCAGCTCTCGGAGGGCGAAGAATCTCGTGCTTTCAGCTTCGATGTAGGAGGGCGTGGATATGTCCTGCGGGTAAATAGCTGCGCCGATGGTTTCTACAAAGATCGTTATGTTTATCGGCACTTTGCATCGGCCGCGCTCCCGATTCCGGAAGTGCTTGACATTGGGGAATTTAGCGAGAGCCTGACCTATTGCATCTCCCGCCGTGCACAGGGTGTCACGTTGCAAGACCTGCCTGAAACCGAACTGCCCGCTGTTCTGCAGCCGGTCGCGGAGGCCATGGATGCGATCGCTGCGGCCGATCTTAGCCAGACGAGCGGGTTCGGCCCATTCGGACCGCAAGGAATCGGTCAATACACTACATGGCGTGATTTCATATGCGCGATTGCTGATCCCCATGTGTATCACTGGCAAACTGTGATGGACGACACCGTCAGTGCGTCCGTCGCGCAGGCTCTCGATGAGCTGATGCTTTGGGCCGAGGACTGCCCCGAAGTCCGGCACCTCGTGCACGCGGATTTCGGCTCCAACAATGTCCTGACGGACAATGGCCGCATAACAGCGGTCATTGACTGGAGCGAGGCGATGTTCGGGGATTCCCAATACGAGGTCGCCAACATCTTCTTCTGGAGGCCGTGGTTGGCTTGTATGGAGCAGCAGACGCGCTACTTCGAGCGGAGGCATCCGGAGCTTGCAGGATCGCCGCGGCTCCGGGCGTATATGCTCCGCATTGGTCTTGACCAACTCTATCAGAGCTTGGTTGACGGCAATTTCGATGATGCAGCTTGGGCGCAGGGTCGATGCGACGCAATCGTCCGATCCGGAGCCGGGACTGTCGGGCGTACACAAATCGCCCGCAGAAGCGCGGCCGTCTGGACCGATGGCTGTGTAGAAGTACTCGCCGATAGTGGAAACCGACGCCCCAGCACTCGTCCGAGGGCAAAGGAATAGGGTACCTTTAAGACCAATGACTTACAAGGCAGCTGTAGATCTTAGCCACTTTTTAAAAGAAAAGGGGGGACTGGAAGGGCTAATTCACTCCCAACGAAGACAAGATCTGCTTTTTGCTTGTACTGGGTCTCTCTGGTTAGACCAGATCTGAGCCTGGGAGCTCTCTGGCTAACTAGGGAACCCACTGCTTAAGCCTCAATAAAGCTTGCCTTGAGTGCTTCAAGTAGTGTGTGCCCGTCTGTTGTGTGACTCTGGTAACTAGAGATCCCTCAGACCCTTTTAGTCAGTGTGGAAAATCTCTAGCAGTAGTAGTTCATGTCATCTTATTATTCAGTATTTATAACTTGCAAAGAAATGAATATCAGAGAGTGAGAGGAACTTGTTTATTGCAGCTTATAATGGTTACAAATAAAGCAATAGCATCACAAATTTCACAAATAAAGCATTTTTTTCACTGCATTCTAGTTGTGGTTTGTCCAAACTCATCAATGTATCTTATCATGTCTGGCTCTAGCTATCCCGCCCCTAACTCCGCCCATCCCGCCCCTAACTCCGCCCAGTTCCGCCCATTCTCCGCCCCATGGCTGACTAATTTTTTTTATTTATGCAGAGGCCGAGGCCGCCTCGGCCTCTGAGCTATTCCAGAAGTAGTGAGGAGGCTTTTTTGGAGGCCTAGGGACGTACCCAATTCGCCCTATAGTGAGTCGTATTACGCGCGCTCACTGGCCGTCGTTTTACAACGTCGTGACTGGGAAAACCCTGGCGTTACCCAACTTAATCGCCTTGCAGCACATCCCCCTTTCGCCAGCTGGCGTAATAGCGAAGAGGCCCGCACCGATCGCCCTTCCCAACAGTTGCGCAGCCTGAATGGCGAATGGGACGCGCCCTGTAGCGGCGCATTAAGCGCGGCGGGTGTGGTGGTTACGCGCAGCGTGACCGCTACACTTGCCAGCGCCCTAGCGCCCGCTCCTTTCGCTTTCTTCCCTTCCTTTCTCGCCACGTTCGCCGGCTTTCCCCGTCAAGCTCTAAATCGGGGGCTCCCTTTAGGGTTCCGATTTAGTGCTTTACGGCACCTCGACCCCAAAAAACTTGATTAGGGTGATGGTTCACGTAGTGGGCCATCGCCCTGATAGACGGTTTTTCGCCCTTTGACGTTGGAGTCCACGTTCTTTAATAGTGGACTCTTGTTCCAAACTGGAACAACACTCAACCCTATCTCGGTCTATTCTTTTGATTTATAAGGGATTTTGCCGATTTCGGCCTATTGGTTAAAAAATGAGCTGATTTAACAAAAATTTAACGCGAATTTTAACAAAATATTAACGCTTACAATTTAGGTGGCACTTTTCGGGGAAATGTGCGCGGAACCCCTATTTGTTTATTTTTCTAAATACATTCAAATATGTATCCGCTCATGAGACAATAACCCTGATAAATGCTTCAATAATATTGAAAAAGGAAGAGTATGAGTATTCAACATTTCCGTGTCGCCCTTATTCCCTTTTTTGCGGCATTTTGCCTTCCTGTTTTTGCTCACCCAGAAACGCTGGTGAAAGTAAAAGATGCTGAAGATCAGTTGGGTGCACGAGTGGGTTACATCGAACTGGATCTCAACAGCGGTAAGATCCTTGAGAGTTTTCGCCCCGAAGAACGTTTTCCAATGATGAGCACTTTTAAAGTTCTGCTATGTGGCGCGGTATTATCCCGTATTGACGCCGGGCAAGAGCAACTCGGTCGCCGCATACACTATTCTCAGAATGACTTGGTTGAGTACTCACCAGTCACAGAAAAGCATCTTACGGATGGCATGACAGTAAGAGAATTATGCAGTGCTGCCATAACCATGAGTGATAACACTGCGGCCAACTTACTTCTGACAACGATCGGAGGACCGAAGGAGCTAACCGCTTTTTTGCACAACATGGGGGATCATGTAACTCGCCTTGATCGTTGGGAACCGGAGCTGAATGAAGCCATACCAAACGACGAGCGTGACACCACGATGCCTGTAGCAATGGCAACAACGTTGCGCAAACTATTAACTGGCGAACTACTTACTCTAGCTTCCCGGCAACAATTAATAGACTGGATGGAGGCGGATAAAGTTGCAGGACCACTTCTGCGCTCGGCCCTTCCGGCTGGCTGGTTTATTGCTGATAAATCTGGAGCCGGTGAGCGTGGGTCTCGCGGTATCATTGCAGCACTGGGGCCAGATGGTAAGCCCTCCCGTATCGTAGTTATCTACACGACGGGGAGTCAGGCAACTATGGATGAACGAAATAGACAGATCGCTGAGATAGGTGCCTCACTGATTAAGCATTGGTAACTGTCAGACCAAGTTTACTCATATATACTTTAGATTGATTTAAAACTTCATTTTTAATTTAAAAGGATCTAGGTGAAGATCCTTTTTGATAATCTCATGACCAAAATCCCTTAACGTGAGTTTTCGTTCCACTGAGCGTCAGACCCCGTAGAAAAGATCAAAGGATCTTCTTGAGATCCTTTTTTTCTGCGCGTAATCTGCTGCTTGCAAACAAAAAAACCACCGCTACCAGCGGTGGTTTGTTTGCCGGATCAAGAGCTACCAACTCTTTTTCCGAAGGTAACTGGCTTCAGCAGAGCGCAGATACCAAATACTGTTCTTCTAGTGTAGCCGTAGTTAGGCCACCACTTCAAGAACTCTGTAGCACCGCCTACATACCTCGCTCTGCTAATCCTGTTACCAGTGGCTGCTGCCAGTGGCGATAAGTCGTGTCTTACCGGGTTGGACTCAAGACGATAGTTACCGGATAAGGCGCAGCGGTCGGGCTGAACGGGGGGTTCGTGCACACAGCCCAGCTTGGAGCGAACGACCTACACCGAACTGAGATACCTACAGCGTGAGCTATGAGAAAGCGCCACGCTTCCCGAAGAGAGAAAGGCGGACAGGTATCCGGTAAGCGGCAGGGTCGGAACAGGAGAGCGCACGAGGGAGCTTCCAGGGGGAAACGCCTGGTATCTTTATAGTCCTGTCGGGTTTCGCCACCTCTGACTTGAGCGTCGATTTTTGTGATGCTCGTCAGGGGGGCGGAGCCTATGGAAAAACGCCAGCAACGCGGCCTTTTTACGGTTCCTGGCCTTTTGCTGGCCTTTTGCTCACATGTTCTTTCCTGCGTTATCCCCTGATTCTGTGGATAACCGTATTACCGCCTTTGAGTGAGCTGATACCGCTCGCCGCAGCCGAACGACCGAGCGCAGCGAGTCAGTGAGCGAGGAAGCGGAAGAGCGCCCAATACGCAAACCGCCTCTCCCCGCGCGTTGGCCGATTCATTAATGCAGCTGGCACGACAGGTTTCCCGACTGGAAAGCGGGCAGTGAGCGCAACGCAATTAATGTGAGTTAGCTCACTCATTAGGCACCCCAGGCTTTACACTTTATGCTTCCGGCTCGTATGTTGTGTGGAATTGTGAGCGGATAACAATTTCACACAGGAAACAGCTATGACCATGATTACGCCAAGCGCGCAATTAACCCTCACTAAAGGGAACAAAAGCTGGAGCTGCAAGCTT